European Patent Specification EP 4 090 761 B1, published May 8, 2024. Title: A DNA-BASED VOLTMETER FOR ORGANELLES. Applicant: University of Chicago. The sequence listing filed with the application follows.

SEQUENCE LISTING (9 sequences)

SEQ ID NO: 1 - DNA, 38 bp, Artificial Sequence
  Synthetic oligonucleotide.
  misc_feature (38)..(38): 3' voltage-sensing fluorophore.
atcaacactgcacaccagacagcaagatcctatatata

SEQ ID NO: 2 - DNA, 16 bp, Artificial Sequence
  Synthetic oligonucleotide.
  misc_feature (1)..(1): 5' reference label.
ggtgtgcagtgttgat

SEQ ID NO: 3 - DNA, 38 bp, Artificial Sequence
  Synthetic oligonucleotide.
  misc_feature (38)..(38): 3' reference label.
tatatataggatcttgctgtctggtgtgcagtgttgat

SEQ ID NO: 4 - DNA, 22 bp, Artificial Sequence
  Synthetic oligonucleotide.
  misc_feature (1)..(1): 5' membrane-anchoring group.
tatatataggatcttgctgtct

SEQ ID NO: 5 - DNA, 38 bp, Artificial Sequence
  Synthetic oligonucleotide.
  misc_feature (1)..(1): 5' voltage-sensing fluorophore.
tatatataggatcttgcttctgtgcctgcagtgttgat

SEQ ID NO: 6 - DNA, 28 bp, Artificial Sequence
  Synthetic oligonucleotide.
  misc_feature (1)..(1): 5' reference label.
atcaacactgcaggcacagagtctggtg

SEQ ID NO: 7 - DNA, 69 bp, Artificial Sequence
  Synthetic oligonucleotide.
  misc_feature (33)..(34): 2' fluoro modified base
  misc_feature (37)..(39): 2' fluoro modified base
  misc_feature (46)..(48): 2' fluoro modified base
  misc_feature (54)..(54): 2' fluoro modified base
  misc_feature (56)..(62): 2' fluoro modified base
  misc_feature (64)..(64): 2' fluoro modified base
  misc_feature (66)..(69): 2' fluoro modified base
caccagacagcaagatcctatatatagggggaucaauccaagggacccggaaacgcucccuuacacccc

SEQ ID NO: 8 - DNA, 20 bp, Artificial Sequence
  Synthetic oligonucleotide.
gggacatgggaatgcaatag

SEQ ID NO: 9 - DNA, 22 bp, Artificial Sequence
  Synthetic oligonucleotide.
ctcaaggtctgagaatgttccc